European Patent Application EP 4 647 494 A1, published November 12, 2025. Title: POLYPEPTIDE AND USE THEREOF. Applicant: HUNAN JIUDIAN PHARMACEUTICAL CO., LTD. Application CN. The sequence listing filed with the application follows.

SEQUENCE LISTING (99 sequences)

SEQ ID NO: 1 - protein, 25 aa, synthetic construct
  DISULFID 21..25: note = intrachain disulfide bond
GKYGFYTKVFRLKKWIQKVICQFGC

SEQ ID NO: 2 - protein, 25 aa, synthetic construct
  DISULFID 21..25: note = intrachain disulfide bond
GKYGFYSKVFRLKKWIQKVICQFGC

SEQ ID NO: 3 - protein, 25 aa, synthetic construct
  DISULFID 21..25: note = intrachain disulfide bond
GKYGFYKKVFRLKKWIQKVICQFGC

SEQ ID NO: 4 - protein, 25 aa, synthetic construct
  DISULFID 21..25: note = intrachain disulfide bond
GKYGFYLKVFRLKKWIQKVICQFGC

SEQ ID NO: 5 - protein, 25 aa, synthetic construct
  DISULFID 21..25: note = intrachain disulfide bond
GKYGFYWKVFRLKKWIQKVICQFGC

SEQ ID NO: 6 - protein, 25 aa, synthetic construct
  DISULFID 21..25: note = intrachain disulfide bond
GKYGFYEKVFRLKKWIQKVICQFGC

SEQ ID NO: 7 - protein, 25 aa, synthetic construct
  DISULFID 21..25: note = intrachain disulfide bond
GKYGFYTKLFRLKKWIQKVICQFGC

SEQ ID NO: 8 - protein, 25 aa, synthetic construct
  DISULFID 21..25: note = intrachain disulfide bond
GKYGFYTKTFRLKKWIQKVICQFGC

SEQ ID NO: 9 - protein, 25 aa, synthetic construct
  DISULFID 21..25: note = intrachain disulfide bond
GKYGFYTKKFRLKKWIQKVICQFGC

SEQ ID NO: 10 - protein, 25 aa, synthetic construct
  DISULFID 21..25: note = intrachain disulfide bond
GKYGFYTKWFRLKKWIQKVICQFGC

SEQ ID NO: 11 - protein, 25 aa, synthetic construct
  DISULFID 21..25: note = intrachain disulfide bond
GKYGFYTKEFRLKKWIQKVICQFGC

SEQ ID NO: 12 - protein, 25 aa, synthetic construct
  DISULFID 21..25: note = intrachain disulfide bond
GKYGFYTKVFRLKKWINKVICQFGC

SEQ ID NO: 13 - protein, 25 aa, synthetic construct
  DISULFID 21..25: note = intrachain disulfide bond
GKYGFYTKVFRLKKWITKVICQFGC

SEQ ID NO: 14 - protein, 25 aa, synthetic construct
  DISULFID 21..25: note = intrachain disulfide bond
GKYGFYTKVFRLKKWIKKVICQFGC

SEQ ID NO: 15 - protein, 25 aa, synthetic construct
  DISULFID 21..25: note = intrachain disulfide bond
GKYGFYTKVFRLKKWIWKVICQFGC

SEQ ID NO: 16 - protein, 25 aa, synthetic construct
  DISULFID 21..25: note = intrachain disulfide bond
GKYGFYTKVFRLKKWILKVICQFGC

SEQ ID NO: 17 - protein, 25 aa, synthetic construct
  DISULFID 21..25: note = intrachain disulfide bond
GKYGFYTKVFRLKKWIQKVICNFGC

SEQ ID NO: 18 - protein, 25 aa, synthetic construct
  DISULFID 21..25: note = intrachain disulfide bond
GKYGFYTKVFRLKKWIQKVICTFGC

SEQ ID NO: 19 - protein, 25 aa, synthetic construct
  DISULFID 21..25: note = intrachain disulfide bond
GKYGFYTKVFRLKKWIQKVICKFGC

SEQ ID NO: 20 - protein, 25 aa, synthetic construct
  DISULFID 21..25: note = intrachain disulfide bond
GKYGFYTKVFRLKKWIQKVICWFGC

SEQ ID NO: 21 - protein, 25 aa, synthetic construct
  DISULFID 21..25: note = intrachain disulfide bond
GKYGFYTKVFRLKKWIQKVICLFGC

SEQ ID NO: 22 - protein, 25 aa, synthetic construct
  DISULFID 21..25: note = intrachain disulfide bond
GKFGFYTKVFRLKKWIQKVICQFGC

SEQ ID NO: 23 - protein, 25 aa, synthetic construct
  DISULFID 21..25: note = intrachain disulfide bond
GKWGFYTKVFRLKKWIQKVICQFGC

SEQ ID NO: 24 - protein, 25 aa, synthetic construct
  DISULFID 21..25: note = intrachain disulfide bond
GKYGYYTKVFRLKKWIQKVICQFGC

SEQ ID NO: 25 - protein, 25 aa, synthetic construct
  DISULFID 21..25: note = intrachain disulfide bond
GKYGWYTKVFRLKKWIQKVICQFGC

SEQ ID NO: 26 - protein, 25 aa, synthetic construct
  DISULFID 21..25: note = intrachain disulfide bond
GKYGFYTKVYRLKKWIQKVICQFGC

SEQ ID NO: 27 - protein, 25 aa, synthetic construct
  DISULFID 21..25: note = intrachain disulfide bond
GKYGFYTKVWRLKKWIQKVICQFGC

SEQ ID NO: 28 - protein, 25 aa, synthetic construct
  DISULFID 21..25: note = intrachain disulfide bond
GKYGFYTKVFKLKKWIQKVICQFGC

SEQ ID NO: 29 - protein, 25 aa, synthetic construct
  DISULFID 21..25: note = intrachain disulfide bond
GKYGFYTKVFRLRKWIQKVICQFGC

SEQ ID NO: 30 - protein, 25 aa, synthetic construct
  DISULFID 21..25: note = intrachain disulfide bond
GKYGFYTKVFRLKKWLQKLICQFGC

SEQ ID NO: 31 - protein, 25 aa, synthetic construct
  DISULFID 21..25: note = intrachain disulfide bond
GKYGFYTKVFRLKKWIQKIICQFGC

SEQ ID NO: 32 - protein, 25 aa, synthetic construct
  DISULFID 21..25: note = intrachain disulfide bond
GKYGFYTKVFRLKKWIQKVLCQFGC

SEQ ID NO: 33 - protein, 25 aa, synthetic construct
  DISULFID 21..25: note = intrachain disulfide bond
GKYGFYTKVFRLKKWIQKVVCQFGC

SEQ ID NO: 34 - protein, 25 aa, synthetic construct
  DISULFID 21..25: note = intrachain disulfide bond
GKYGFYTKVFRLKKWIQKVTCQFGC

SEQ ID NO: 35 - protein, 25 aa, synthetic construct
  DISULFID 21..25: note = intrachain disulfide bond
GKYGFYTKVFRLKKWIQKVICQYGC

SEQ ID NO: 36 - protein, 25 aa, synthetic construct
  DISULFID 21..25: note = intrachain disulfide bond
GKYGFYTKVFRLKKWIQKVICQWGC

SEQ ID NO: 37 - protein, 25 aa, synthetic construct
  DISULFID 21..25: note = intrachain disulfide bond
  SITE 21: note = D-Cysteine
GKYGFYTKVFRLKKWIQKVIXQFGC

SEQ ID NO: 38 - protein, 25 aa, synthetic construct
  DISULFID 21..25: note = intrachain disulfide bond
  SITE 25: note = D-Cysteine
GKYGFYTKVFRLKKWIQKVICQFGX

SEQ ID NO: 39 - protein, 25 aa, synthetic construct
  DISULFID 21..25: note = intrachain disulfide bond
  SITE 21: note = D-Cysteine
  SITE 25: note = D-Cysteine
GKYGFYTKVFRLKKWIQKVIXQFGX

SEQ ID NO: 40 - protein, 25 aa, synthetic construct
GKYGFYTKVFRLKKWIQKVIKQFGE

SEQ ID NO: 41 - protein, 25 aa, synthetic construct
GKYGFYTKVFRLKKWIQKVIDQFGK

SEQ ID NO: 42 - protein, 25 aa, synthetic construct
GKYGFYTKVFRLKKWIQKVIKQFGK

SEQ ID NO: 43 - protein, 25 aa, synthetic construct
GKYGFYTKVFRLKKWIQKVILQFGE

SEQ ID NO: 44 - protein, 25 aa, synthetic construct
GKYGFYTKVFRLKKWIQKVIWQFGE

SEQ ID NO: 45 - protein, 25 aa, synthetic construct
GKYGFYTKVFRLKKWIQKVISQFGE

SEQ ID NO: 46 - protein, 25 aa, synthetic construct
GKYGFYTKVFRLKKWIQKVIDQFGL

SEQ ID NO: 47 - protein, 25 aa, synthetic construct
GKYGFYTKVFRLKKWIQKVIDQFGW

SEQ ID NO: 48 - protein, 25 aa, synthetic construct
GKYGFYTKVFRLKKWIQKVIDQFGS

SEQ ID NO: 49 - protein, 25 aa, synthetic construct
  DISULFID 21..25: note = intrachain disulfide bond
GKYGFYTRVFRLKKWIQKVICQFGC

SEQ ID NO: 50 - protein, 25 aa, synthetic construct
  DISULFID 21..25: note = intrachain disulfide bond
GKWGWYTKVFRLKKWIQKVICQFGC

SEQ ID NO: 51 - protein, 25 aa, synthetic construct
  DISULFID 21..25: note = intrachain disulfide bond
GKWGWYWKVFRLKKWIQKVICQFGC

SEQ ID NO: 52 - protein, 25 aa, synthetic construct
  DISULFID 21..25: note = intrachain disulfide bond
GKWGFYWKVFRLKKWIQKVICQFGC

SEQ ID NO: 53 - protein, 25 aa, synthetic construct
  DISULFID 21..25: note = intrachain disulfide bond
GKWGWYWRVFRLKKWIQKVICQFGC

SEQ ID NO: 54 - protein, 25 aa, synthetic construct
  DISULFID 21..25: note = intrachain disulfide bond
GKWGWYWRLFRLKKWIQKVICQFGC

SEQ ID NO: 55 - protein, 25 aa, synthetic construct
  DISULFID 21..25: note = intrachain disulfide bond
GKWGWYWRLWRLKKWIQKVICQFGC

SEQ ID NO: 56 - protein, 25 aa, synthetic construct
  DISULFID 21..25: note = intrachain disulfide bond
GKWGWYWRLWKLKKWIQKVICQFGC

SEQ ID NO: 57 - protein, 25 aa, synthetic construct
  DISULFID 21..25: note = intrachain disulfide bond
GKWGWYWRLWKLRKWIQKVICQFGC

SEQ ID NO: 58 - protein, 25 aa, synthetic construct
  DISULFID 21..25: note = intrachain disulfide bond
GKWGWYWRLWKLRKWIWKVICQFGC

SEQ ID NO: 59 - protein, 25 aa, synthetic construct
  DISULFID 21..25: note = intrachain disulfide bond
GKWGWYWRLWKLRKWILKVICQFGC

SEQ ID NO: 60 - protein, 25 aa, synthetic construct
  DISULFID 21..25: note = intrachain disulfide bond
GKWGWYWRLWKLRKWIWKLICQFGC

SEQ ID NO: 61 - protein, 25 aa, synthetic construct
  DISULFID 21..25: note = intrachain disulfide bond
GKWGWYWRLWKLRKWIWKLLCQFGC

SEQ ID NO: 62 - protein, 25 aa, synthetic construct
  DISULFID 21..25: note = intrachain disulfide bond
GKWGWYWRLWKLRKWIWKLLCTFGC

SEQ ID NO: 63 - protein, 25 aa, synthetic construct
  DISULFID 21..25: note = intrachain disulfide bond
GKWGWYWRLWKLRKWIWKLLCTWGC

SEQ ID NO: 64 - protein, 25 aa, synthetic construct
  DISULFID 21..25: note = intrachain disulfide bond
GKWGWYWRLWKLRKWILKLLCTWGC

SEQ ID NO: 65 - protein, 25 aa, synthetic construct
  DISULFID 21..25: note = intrachain disulfide bond
GKWGWYWRLWKLRKWILKLLCWWGC

SEQ ID NO: 66 - protein, 25 aa, synthetic construct
  DISULFID 21..25: note = intrachain disulfide bond
GKWGWYWRKWKLRKWIWKLLCTWGC

SEQ ID NO: 67 - protein, 25 aa, synthetic construct
  DISULFID 21..25: note = intrachain disulfide bond
GKWGFYTRVFRLKKWIQKVICQWGC

SEQ ID NO: 68 - protein, 25 aa, synthetic construct
  DISULFID 21..25: note = intrachain disulfide bond
GKWGFYWRVFRLKKWIQKVICQWGC

SEQ ID NO: 69 - protein, 25 aa, synthetic construct
  DISULFID 21..25: note = intrachain disulfide bond
GKWGFYTRVFRLKKWIQKVICTWGC

SEQ ID NO: 70 - protein, 25 aa, synthetic construct
  DISULFID 21..25: note = intrachain disulfide bond
GKWGFYTRVFRLKKWIWKVICTWGC

SEQ ID NO: 71 - protein, 25 aa, synthetic construct
  DISULFID 21..25: note = intrachain disulfide bond
GKWGFYTRVFRLKKWILKVICTWGC

SEQ ID NO: 72 - protein, 25 aa, synthetic construct
  DISULFID 21..25: note = intrachain disulfide bond
GKWGFYTRVFRLKKWIWKLLCTWGC

SEQ ID NO: 73 - protein, 25 aa, synthetic construct
  DISULFID 21..25: note = intrachain disulfide bond
GKWGWYWRVFRLKKWIWKVICTWGC

SEQ ID NO: 74 - protein, 25 aa, synthetic construct
  DISULFID 21..25: note = intrachain disulfide bond
GKWGFYTKVFRLKKWIQKVICQFGC

SEQ ID NO: 75 - protein, 25 aa, synthetic construct
  DISULFID 21..25: note = intrachain disulfide bond
GKWGFYTKVFRLKKWIQKVICQFGC

SEQ ID NO: 76 - protein, 25 aa, synthetic construct
  DISULFID 21..25: note = intrachain disulfide bond
GKWGFYTKVFRLKKWIQKVICQFGC

SEQ ID NO: 77 - protein, 25 aa, synthetic construct
  DISULFID 21..25: note = intrachain disulfide bond
GKWGFYTKVFRLKKWIQKVICTWGC

SEQ ID NO: 78 - protein, 25 aa, synthetic construct
  DISULFID 21..25: note = intrachain disulfide bond
GKWGFYTKKFRLKKWIQKVICQFGC

SEQ ID NO: 79 - protein, 25 aa, synthetic construct
  DISULFID 21..25: note = intrachain disulfide bond
GKWGFYTKKFRLKKWIQKVICTWGC

SEQ ID NO: 80 - protein, 25 aa, synthetic construct
  DISULFID 21..25: note = intrachain disulfide bond
GKWGFYTKVFRLKKWIQKVICTFGC

SEQ ID NO: 81 - protein, 25 aa, synthetic construct
  DISULFID 21..25: note = intrachain disulfide bond
GKWGFYTKVFRLKKWIQKVICQWGC

SEQ ID NO: 82 - protein, 25 aa, synthetic construct
  DISULFID 21..25: note = intrachain disulfide bond
GKWGFYTKKFRLKKWIQKVICTFGC

SEQ ID NO: 83 - protein, 25 aa, synthetic construct
  DISULFID 21..25: note = intrachain disulfide bond
GKWGFYTKKFRLKKWIQKVICQWGC

SEQ ID NO: 84 - protein, 25 aa, synthetic construct
  DISULFID 21..25: note = intrachain disulfide bond
GKWGFYTKRFRLKKWIQKVICTWGC

SEQ ID NO: 85 - protein, 25 aa, synthetic construct
  DISULFID 21..25: note = intrachain disulfide bond
GKWGFYTRKFRLKKWIQKVICTWGC

SEQ ID NO: 86 - protein, 25 aa, synthetic construct
  DISULFID 21..25: note = intrachain disulfide bond
GKWGFYTKVFRLKKWIQKVICTWGC

SEQ ID NO: 87 - protein, 25 aa, synthetic construct
  DISULFID 21..25: note = intrachain disulfide bond
GKWGFYTKVFRLKKWIQKVICTFGC

SEQ ID NO: 88 - protein, 25 aa, synthetic construct
  DISULFID 21..25: note = intrachain disulfide bond
GKWGFYTKVFRLKKWILKVICTWGC

SEQ ID NO: 89 - protein, 25 aa, synthetic construct
  DISULFID 21..25: note = intrachain disulfide bond
GKWGFYTKVFRLKKWILKVICTFGC

SEQ ID NO: 90 - protein, 25 aa, synthetic construct
  DISULFID 21..25: note = intrachain disulfide bond
GKWGFYTKVFRLKKWIIKVICTFGC

SEQ ID NO: 91 - protein, 25 aa, synthetic construct
  DISULFID 21..25: note = intrachain disulfide bond
GKWGFYTKVFRLKKWIVKVICTFGC

SEQ ID NO: 92 - protein, 25 aa, synthetic construct
  DISULFID 21..25: note = intrachain disulfide bond
GKWGFYTKVFRLKKWIWKVICTFGC

SEQ ID NO: 93 - protein, 25 aa, synthetic construct
  DISULFID 21..25: note = intrachain disulfide bond
GKWGFYTKVFRLKKWIFKVICTFGC

SEQ ID NO: 94 - protein, 25 aa, synthetic construct
  DISULFID 21..25: note = intrachain disulfide bond
GKWGFYTKVFRLKKWIYKVICTFGC

SEQ ID NO: 95 - protein, 25 aa, synthetic construct
  DISULFID 21..25: note = intrachain disulfide bond
GKWGFYTKVFRLKKWIKKVICTFGC

SEQ ID NO: 96 - protein, 25 aa, synthetic construct
  DISULFID 21..25: note = intrachain disulfide bond
GKWGFYTKVFRLKKWIRKVICTFGC

SEQ ID NO: 97 - protein, 25 aa, synthetic construct
  DISULFID 21..25: note = intrachain disulfide bond
GKWGFYTKVFRLKKWIMKVICTFGC

SEQ ID NO: 98 - protein, 25 aa, synthetic construct
  DISULFID 21..25: note = intrachain disulfide bond
GKWGFYTKVFRLKKWINKVICTFGC

SEQ ID NO: 99 - protein, 25 aa, synthetic construct
  DISULFID 21..25: note = intrachain disulfide bond
GKWGFYTKVFRLKKWISKVICTFGC